European Patent Application EP 4 722 376 A2, published April 8, 2026. Title: CHIMERIC TERMINAL DEOXYNUCLEOTIDYL TRANSFERASES FOR TEMPLATE-FREE ENZYMATIC SYNTHESIS OF POLYNUCLEOTIDES. Applicant: DNA SCRIPT. The sequence listing filed with the application follows.

SEQUENCE LISTING (83 sequences)

SEQ ID NO: 1 - protein, 510 aa, synthetic construct
  REGION 1..510: note = Full length wild type mouse TdT
MDPLQAVHLGPRKKRPRQLGTPVASTPYDIRFRDLVLFILEKKMGTTRRAFLMELARRKGFRVENELSDSVTHIVAENNSGSDVLEWLQLQNIKASSELELLDISWLIECMGAGKPVEMMGRHQLVVNRNSSPSPVPGSQNVPAPAVKKISQYACQRRTTLNNYNQLFTDALDILAENDELRENEGSCLAFMRASSVLKSLPFPITSMKDTEGIPCLGDKVKSIIEGIIEDGESSEAKAVLNDERYKSFKLFTSVFGVGLKTAEKWFRMGFRTLSKIQSDKSLRFTQMQKAGFLYYEDLVSCVNRPEAEAVSMLVKEAVVTFLPDALVTMTGGFRRGKMTGHDVDFLITSPEATEDEEQQLLHKVTDFWKQQGLLLYCDILESTFEKFKQPSRKVDALDHFQKCFLILKLDHGRVHSEKSGQQEGKGWKAIRVDLVMCPYDRRAFALLGWTGSRQFERDLRRYATHERKMMLDNHALYDRTKRVFLEAESEEEIFAHLGLDYIEPWERNA

SEQ ID NO: 2 - protein, 381 aa, synthetic construct
  REGION 1..381: note = truncated wild type mouse TdT
NSSPSPVPGSQNVPAPAVKKISQYACQRRTTLNNYNQLFTDALDILAENDELRENEGSCLAFMRASSVLKSLPFPITSMKDTEGIPCLGDKVKSIIEGIIEDGESSEAKAVLNDERYKSFKLFTSVFGVGLKTAEKWFRMGFRTLSKIQSDKSLRFTQMQKAGFLYYEDLVSCVNRPEAEAVSMLVKEAVVTFLPDALVTMTGGFRRGKMTGHDVDFLITSPEATEDEEQQLLHKVTDFWKQQGLLLYCDILESTFEKFKQPSRKVDALDHFQKCFLILKLDHGRVHSEKSGQQEGKGWKAIRVDLVMCPYDRRAFALLGWTGSRQFERDLRRYATHERKMMLDNHALYDRTKRVFLEAESEEEIFAHLGLDYIEPWERNA

SEQ ID NO: 3 - protein, 380 aa, synthetic construct
  REGION 1..380: note = Bovine truncated
DYSATPNPGFQKTPPLAVKKISQYACQRKTTLNNYNHIFTDAFEILAENSEFKENEVSYVTFMRAASVLKSLPFTIISMKDTEGIPCLGDKVKCIIEEIIEDGESSEVKAVLNDERYQSFKLFTSVFGVGLKTSEKWFRMGFRSLSKIMSDKTLKFTKMQKAGFLYYEDLVSCVTRAEAEAVGVLVKEAVWAFLPDAFVTMTGGFRRGKKIGHDVDFLITSPGSAEDEEQLLPKVINLWEKKGLLLYYDLVESTFEKFKLPSRQVDTLDHFQKCFLILKLHHQRVDSSKSNQQEGKTWKAIRVDLVMCPYENRAFALLGWTGSRQFERDIRRYATHERKMMLDNHALYDKTKRVFLKAESEEEIFAHLGLDYIEPWERNA

SEQ ID NO: 4 - protein, 380 aa, synthetic construct
  REGION 1..380: note = Human truncated
DYSDSTNPGPPKTPPIAVQKISQYACQRRTTLNNCNQIFTDAFDILAENCEFRENEDSCVTFMRAASVLKSLPFTIISMKDTEGIPCLGSKVKGIIEEIIEDGESSEVKAVLNDERYQSFKLFTSVFGVGLKTSEKWFRMGFRTLSKVRSDKSLKFTRMQKAGFLYYEDLVSCVTRAEAEAVSVLVKEAVWAFLPDAFVTMTGGFRRGKKMGHDVDFLITSPGSTEDEEQLLQKVMNLWEKKGLLLYYDLVESTFEKLRLPSRKVDALDHFQKCFLIFKLPRQRVDSDQSSWQEGKTWKAIRVDLVLCPYERRAFALLGWTGSRQFERDLRRYATHERKMILDNHALYDKTKRIFLKAESEEEIFAHLGLDYIEPWERNA

SEQ ID NO: 5 - protein, 376 aa, synthetic construct
  REGION 1..376: note = Chicken truncated
QYPTLKTPESEVSSFTASKVSQYSCQRKTTLNNCNKKFTDAFEIMAENYEFKENEIFCLEFLRAASVLKSLPFPVTRMKDIQGLPCMGDRVRDVIEEIIEEGESSRAKDVLNDERYKSFKEFTSVFGVGVKTSEKWFRMGLRTVEEVKADKTLKLSKMQRAGFLYYEDLVSCVSKAEADAVSSIVKNTVCTFLPDALVTITGGFRRGKKIGHDIDFLITSPGQREDDELLHKGLLLYCDIIESTFVKEQIPSRHVDAMDHFQKCFAILKLYQPRVDNSSYNMSKKCDMAEVKDWKAIRVDLVITPFEQYAYALLGWTGSRQFGRDLRRYATHERKMMLDNHALYDKRKRVFLKAGSEEEIFAHLGLDYVEPWERNA

SEQ ID NO: 6 - protein, 387 aa, synthetic construct
  REGION 1..387: note = Possum truncated
SANPDPTAGTLNILPPTTKTISQYACQRRTTINNHNQRFTDAFEILAKNYEFKENDDTCLTFMRAISVLKCLPFEVVSLKDTEGLPWIGDEVKGIMEEIIEDGESLEVQAVLNDERYQSFKLFTSVFGVGLKTADKWYRMGFRTLNKIRSDKTLKLTKMQKAGLCYYEDLIDCVSKAEADAVSLLVQDAVWTFLPDALVTITGGFRRGKEFGHDVDFLITSPGAEKEQEDQLLQKVTNLWKKQGLLLYCDLIESTFEDLKLPSRKIDALDHFQKCFLILKLYHHKEDKRKWEMPTGSNESEAKSWKAIRVDLVVCPYDRYAFALLGWSGSRQFERDLRRYATHEKKMMLDNHALYDKTKKIFLKAKSEEEIFAHLGLEYIQPSERNA

SEQ ID NO: 7 - protein, 381 aa, synthetic construct
  REGION 1..381: note = New truncated shrew
DCPASHDSSPQKTESAAVQKISQYACQRRTTLNNHNHIFTDAFEILAENCEFRENEGSYVTYMRAASVLKSLPFSIISMKDTEGIPCLADKVKCVIEEIIEDGESSEVKAVLNDERYKSFKLFTSVFGVGLKTAEKWFRLGFRTLSGIMNDKTLKLTHMQKAGFLYYEDLVSCVTRAEAEAVGVLVKEAVWAFLPDAIVTMTGGFRRGKKVGHDVDFLITSPEATEEQEQQLLHKVITFWEKEGLLLYCDLYESTFEKLKMPSRKVDALDHFQKCFLILKLHRECVDDGTSSQLQGKTWKAIRVDLVVCPYECRAFALLGWTGSPQFERDLRRYATHERKMMLDNHALYDKTKRKFLSADSEEDIFAHLGLDYIEPWERNA

SEQ ID NO: 8 - protein, 381 aa, synthetic construct
  REGION 1..381: note = truncated dog
DYTASPNPELQKTLPVAVKKISQYACQRRTTLNNYNNVFTDAFEVLAENYEFRENEVFSLTFMRAASVLKSLPFTIISMKDTEGIPCLGDQVKCIIEEIIEDGESSEVKAVLNDERYQSFKLFTSVFGVGLKTSEKWFRMGFRTLSKIKSDKSLKFTPMQKAGFLYYEDLVSCVTRAEAEAVGVLVKEAVGAFLPDAFVTMTGGFRRGKKMGHDVDFLITSPGSTDEDEEQLLPKVINLWERKGLLLYCDLVESTFEKLKLPSRKVDALDHFQKCFLILKLHHQRVDGGKCSQQEGKTWKAIRVDLVMCPYERRAFALLGWTGSRQFERDLRRYASHERKMILDNHALYDKTKKIFLKAESEEEIFAHLGLDYIEPWERNA

SEQ ID NO: 9 - protein, 382 aa, synthetic construct
  REGION 1..382: note = TRUNC MOLE
GDCPASHDSSPQKTESAAVQKISQYACQRRTTLNNHNHIFTDAFEILAENCEFRENEGSYVTYMRAASVLKSLPFSIISMKDTEGIPCLADKVKCVIEEIIEDGESSEVKAVLNDERYKSFKLFTSVFGVGLKTAEKWFRLGFRTLSGIMNDKTLKLTHMQKAGFLYYEDLVSCVTRAEAEAVGVLVKEAVWAFLPDAIVTMTGGFRRGKKVGHDVDFLITSPEATEEQEQQLLHKVITFWEKEGLLLYCDLYESTFEKLKMPSRKVDALDHFQKCFLILKLHRECVDDGTSSQLQGKTWKAIRVDLVVCPYECRAFALLGWTGSPQFERDLRRYATHERKMMLDNHALYDKTKRKFLSADSEEDIFAHLGLDYIEPWERNA

SEQ ID NO: 10 - protein, 379 aa, synthetic construct
  REGION 1..379: note = Pika truncated
EYSANPSPGPQATPAVYKISQYACQRRTTLNNHNHIFTDAFEILAENYEFKENEGCYVTYMRAASVLKSLPFTIVSMKDTEGIPCLEDKVKSIMEEIIEEGESSEVKAVLSDERYQCFKLFTSVFGVGLKTSEKWFRMGFRSLSNIRLDKSLKFTQMQKAGFRYYEDIVSCVTRAEAEAVDVLVNEAVRAFLPDAFITMTGGFRRGKKIGHDVDFLITSPELTEEDEQQLLHKVMNLWEKKGLLLYHDLVESTFEKLKQPSRKVDALDHFQKCFLIFKLYHERVGGDRCRQPEGKDWKAIRVDLVMCPYECHAFALLGWTGSRQFERDLRRYASHERKMILDNHALYDKTKRVFLQAENEEEIFAHLGLDYIEPWERNA

SEQ ID NO: 11 - protein, 384 aa, synthetic construct
  REGION 1..384: note = TRUNC HEDGEHOG
DASFGSNPGSQNTPPLAIKKISQYACQRRTSLNNCNHIFTDALDILAENHEFRENEVSCVAFMRAASVLKSLPFTIISMKDTKGIPCLGDKAKCVIEEIIEDGESSEVKAILNDERYQSFKLFTSVFGVGLKTSEKWFRMGFRTLNKIMSDKTLKLTRMQKAGFLYYEDLVSCVAKAEADAVSVLVQEAVWAFLPDAMVTMTGGFRRGKKLGHDVDFLITSPGATEEEEQQLLPKVINFWERKGLLLYHDLVESTFEKLKLPSRKVDALDHFQKCFLILKLHLQHVNGVGNSKTGQQEGKNWKAIRVDLVMCPYERRAFALLGWTGSRQFERDLRRFATHERKMMLDNHALYDKTKRIFLKAESEEEIFAHLGLDYIDPWERNA

SEQ ID NO: 12 - protein, 381 aa, synthetic construct
  REGION 1..381: note = truncated tree shrew
DHSTSPSPGPQKTPALAVQKISQYACQRRTTLNNCNRVFTDAFETLAENYEFRENEDSSVIFLRAASVLRSLPFTITSMRDTEGLPCLGDKVKCVIEEIIEDGESSEVNAVLNDERYKSFKLFTSVFGVGLKTSEKWFRMGFRTLSRVRSDKSLHLTRMQQAGFLYYEDLASCVTRAEAEAVGVLVKEAVGAFLPDALVTITGGFRRGKKTGHDVDFLITSPGSTEEKEEELLQKVLNLWEKKGLLLYYDLVESTFEKLKTPSRKVDALDHFPKCFLILKLHHQRVDGDKPSQQEGKSWKAIRVDLVMCPYERHAFALLGWTGSRQFERDLRRYATHERKMMLDNHALYDKTKRVFLKAESEEDIFAHLGLDYIEPWERNA

SEQ ID NO: 13 - protein, 394 aa, synthetic construct
  REGION 1..394: note = TRUNCATED PLATYPUS
LTNSAPINCMTETPSLATKQVSQYACERRTTLNNCNQKFTDAFEILAKDFEFRENEGICLAFMRAISVLKCLPFTIVRMKDIEGVPWLGDQVKSIIEEIIEDGESSSVKAVLNDERYRSFQLFNSVFEVGLTDNGENGIARGFQTLNEVITDENISLTKTTLSTSLWNYLPGFLYYEDLVSCVAKEEADAVYLIVKEAVRAFLPEALVTLTGGFRRGKKIGHDVDFLISDPESGQDEQLLPNIIKLWEKQELLLYYDLVESTFEKTKIPSRKVDAMDHFQKCFLILKLHHQKVDSGRYKPPPESKNHEAKNWKAIRVDLVMCPFEQYAYALLGWTGSRQFERDLRRYATHEKKMMLDNHALYDKTKKIFLKAESEEDIFTHLGLDYIEPWERNA

SEQ ID NO: 14 - protein, 384 aa, synthetic construct
  REGION 1..384: note = TRUNCATED JERBOA
SSELELLDVSWLIECMGAGKPVEMTGRHQLVKQTFCLPGFILQDAFDILAENCEFRENEASCVEFMRAASVLKSLPFPIISVKDTEGIPWLGGKVKCVIEEIIEDGESSEVKALLNDERYKSFKLFTSVFGVGLKTAERWFRMGFRTLSTVKLDKSLTFTRMQKAGFLHYEDLVSCVTRAEAEAVSVLVQQAVVAFLPDALVSMTGGFRRGKKIGHDVDFLITSPEATEEEEQQLLHKVTNFWEQKGLLLYCDHVESTFEKCKLPSRKVDALDHFQKCFLILKLYRERVDSVKSSQQEGKGWKAIRVDLVMCPYECRAFALLGWTGSRQFERDLRRYATHERKMRLDNHALYDKTKRVFLKAESEEEIFAHLGLEYIEPLERNA

SEQ ID NO: 15 - protein, 364 aa, synthetic construct
  REGION 1..364: note = Puma wildtype
VVKKIPLYACQRRTTLNNFNHIFTDAFEVLAENYEFKENEISSATFMRAASVLKLPFTIISMKDTEGIPCLGDKVKCVIEEIIEDGESSEVKAVLNDERYQSFKLFTSVFGVGLKTSEKWFRMGFRTLSKIKSDKTLKFTQMQKAGFLYYEDLVSCVTRAEAEAVGVLVKEAVWAFLPDAFVTMTGGFRRGKKIGHDVDFLITIPGSTDEEEEQLLPKVINLWQRKELLLYYDLVESTFEKLKLPSRKVDALDHFQKCFLILKLHHQRVDSGKCSQQEGKTWKAIRVDLVMCPYERRAFALLGWTGSRQFERDLRRYATHERKMILDNHALYDKTKKIFLKAESEEEIFAHLGLDYIEPWERNA

SEQ ID NO: 16 - DNA, 12 bp, synthetic construct
  misc_feature 1..12: note = Test Polynucleotide p875
  source 1..12: mol_type = other DNA
cagttaaaaact

SEQ ID NO: 17 - DNA, 11 bp, synthetic construct
  misc_feature 1..11: note = Test Polynucleotide p876
  source 1..11: mol_type = other DNA
gagttaaaact

SEQ ID NO: 18 - DNA, 10 bp, synthetic construct
  misc_feature 1..10: note = Test Polynucleotide p877
  source 1..10: mol_type = other DNA
cagcaaggct

SEQ ID NO: 19 - protein, 25 aa, synthetic construct
  REGION 1..25: note = HIS-TAG
MASSHHHHHHSSGSENLYFQTGSSG

SEQ ID NO: 20 - DNA, 18 bp, synthetic construct
  misc_feature 1..18: note = PRIMER
  source 1..18: mol_type = other DNA
aaaaaaaaaaaaaagggg

SEQ ID NO: 21 - protein, 381 aa, synthetic construct
  REGION 1..381: note = Truncated mouse TdT M53
NSSPSPVPGSQNAPAPVVKKISQYACQRRTTLNNYNELFTRALDILAENDEFRENEESRDAFRRASSVLKSLPFPITSMKDTEGIPCLGDKVKRIIEEIIEDGESSEVKAVLNDERYKAFKLFTSVFGVGRKTAEKWFRMGFRTLEKIRSDKSLRFTQMQKAGFLYYEDLAERVNRPEAEAIRMLVKEAVVTFLPDALVTMTGGFRLGKMTGHDVDFLITSPEATEDEEQQLLHKVTDFWKQQGLLLYCDILESTFEKFKQPSRTVDALDHFQKCFLILKLDHPRVHSVKSGQQEGKGWKAIRVDLVMCPYDRRAFALLGWTGSPQFNRDLRRYATHERKMMLDNHALYDKTKRVFLEAESEEEIFAHLGLDYIEPWERNA

SEQ ID NO: 22 - protein, 369 aa, synthetic construct
  REGION 1..369: note = TRUNCATED BOVINE
KTPPLVVKKISQYACQRKTTLNNYNEIFTRAFEILAENSEFKENEESYVTFRRAASVLKSLPFTIISMKDTEGIPCLGDKVKRIIEEIIEDGESSEVKAVLNDERYQAFKLFTSVFGVGRKTSEKWFRMGFRSLEKIRSDKTLKFTKMQKAGFLYYEDLVSGVTRAEAEAVGVLVKEAVWAFLPDAFVTMTGGFRLGKKIGHDVDFLITSPGSAEDEEQLLPKVINLWEKKGLLLYYDLVESTFEKFKLPSRQVDTLDHFQKCFLILKLHHQRVDSSKSNQQEGKTWKAIRVDLVMCPYENRAFALLGWTGSAFFNRDIRRYATHERKMMLDNHALYDKTKRVFLKAESEEEIFAHLGLDYIEPRERNA

SEQ ID NO: 23 - protein, 378 aa, synthetic construct
  REGION 1..378: note = M57 without His tag & linker
SPSPVPGSQNAPAPVVKKISQYACQRRTTLNNYNELFTRALDILAENDEFRENEESRDAFRRASSVLKSLPFPITSMKDTEGIPCLGDKVKRIIEEIIEDGESSEVKAVLNDERYKAFKLFTSVFGVGRKTAEKWFRMGFRTLEKIRSDKSLRFTQMQKAGFLYYEDLVSGVTRAEAEAVGVLVKEAVWAFLPDAFVTMTGGFRLGKKIGHDVDFLITSPGSAEDEEQLLPKVINLWEKKGLLLYYDLVESTFEKFKLPSRQVDTLDHFQKCFLILKLHHQRVDSSKSNQQEGKTWKAIRVDLVMCPYENRAFALLGWTGSPQFNRDLRRYATHERKMMLDNHALYDKTKRVFLEAESEEEIFAHLGLDYIEPWERNA

SEQ ID NO: 24 - protein, 378 aa, synthetic construct
  REGION 1..378: note = M59 without His Tag and linker
SPSPVPGSQNAPAPVVKKISQYACQRRTTLNNYNELFTRALDILAENDEFRENEESRDAFRRASSVLKSLPFPITSMKDTEGIPCLGDKVKRIIEEIIEDGESSEVKAVLNDERYKAFKLFTSVFGVGRKTAEKWFRMGFRTLEKIRSDKSLRFTQMQKAGFLYYEDLAERVNRPEAEAIRMLVKEAVVTFLPDALVTMTGGFRLGKMTGHDVDFLITSPGSAEDEEQLLPKVINLWEKKGLLLYYDLVESTFEKFKLPSRQVDTLDHFQKCFLILKLHHQRVDSSKSNQQEGKTWKAIRVDLVMCPYENRAFALLGWTGSPQFNRDLRRYATHERKMMLDNHALYDKTKRVFLEAESEEEIFAHLGLDYIEPWERNA

SEQ ID NO: 25 - protein, 381 aa, synthetic construct
  REGION 1..381: note = M27
NSSPSPVPGSQNVPAPVVKKISQYACQRRTTLNNYNQLFTDALDILAENDEFRENEESCLAFRRASSVLKSLPFPITSMKDTEGIPCLGDKVKSIIEGIIEDGESSEVKAVLNDERYKSFKLFTSVFGVGLKTAEKWFRMGFRTLSKIQSDKSLRFTQMQKAGFLYYEDLVSGVNRPEAEAVSMLVKEAVVTFLPDALVTMTGGFRLGKMTGHDVDFLITSPEATEDEEQQLLHKVTDFWKQQGLLLYCDILESTFEKFKQPSRTVDALDHFQKCFLILKLDHPRVHSVKSGQQEGKGWKAIRVDLVMCPYDRRAFALLGWTGSPQFNRDLRRYATHERKMMLDNHALYDKTKRVFLEAESEEEIFAHLGLDYIEPWERNA

SEQ ID NO: 26 - protein, 382 aa, synthetic construct
  REGION 1..382: note = B10 trunc wt (Serinus canaria)(canary)
SPPLNTPELEMPSFIATKVSQYSCQRKTTLNNYNKKFTDAFEVMAENYEFKENEIFCLEFLRAASLLKSLPFSVTRMKDIQGLPCMGDQVRDVIEIIEEGESSRVKEVLNDERYKAFKQFTSVFGVGVKTSEKWYRMGLRTVGEVKADKTLKLSKMQKAGFLYYEDLVSCVSKAEADAVSLIVKNTVCTFLPDALVTITGGFRRGKNIGHDIDFLITNPGPREDDELLHKVIDLWKKQGLLLYCDIIESTFVKEQLPSRKIDAMDHFQKCFAILKLYQPRVDNSTCNTSKKLEMAEVKDWKAIRVDLVITPFEQYSYALLGWTGSRQFGRDLRRYAAHERRMILDNHGLYDRTKRIFLKAGSEEEIFAHLGLDYVEPWERNA

SEQ ID NO: 27 - protein, 370 aa, synthetic construct
  REGION 1..370: note = B19 trunc wt (Neopelma chrysocephalum)(saffron-crested neopelma)
FIARKVSQYSCQRKTTLNNYNKKFTDAFEIMAENYEFKENEIFCLEFLRAASLLKYLPFPVTRMKDIQGLPCIGDQVRDVIEGIIEEGESSRVKEVLNDERYKAFKQFTSVFGVGVKTSEKWYRMGLRTVEELKADKTLKLSKMQKAGFLYYEDLVSCVSKAEADAVTLIVKNTVSTFLPDALVTITGGFRRGKKMGHDIDFLITNPGPREDDELLHKVVDLWKKQGLLLYCDIIESTFVEEQLPSRKVDAMDNFQKCFTILKLYQPGVDNSSYNMSKKSDMAEVKDWKAIRVDLVITPFEQYAYALLGWTGSREFGRDLRRYASHERKMILDNHGLYDRRKRIFLKAGSEEEIFAHLGLDYVEPWERNA

SEQ ID NO: 28 - protein, 383 aa, synthetic construct
  REGION 1..383: note = trunc wt (Alligator sinensis)
SPSPVPGSQNVPAPSVDKVSQYACQRRTTLNNYNKKFTDAFEILAENCEFRENRLGCLEFLRAASVLKFLPFPIVKMKNIEGLPCMGDKVKCVIEEILEEGESCQAKEILNDERYKSFKLFTSVFGVGLKTTEKWYRMGFRTLEEVKAEKTLKLSRMQIAGFLHYEDIISYVSKAEADAVSLLIKDTVCMFLPDALVTITGGFRRGKKTGHDVDFLITNPGPEEEKELLHKVVDLWEKQGLLLYYDVIESTFEKEKRPSRKVDALDHFQKCFAILKLHQQRRGNSNSNISKESDKAEVKDWKAIRVDLVISPFEQYAYALLGWTGSRQFERDLRRYASRERKMMLDNHALYDKTKRTFLKAESEEEIFAHLGLDYIEPWERNA

SEQ ID NO: 29 - protein, 380 aa, synthetic construct
  REGION 1..380: note = B59 trunc wt (Xenopus laevis)
SPSPVPGSQNVPAPSEVKVSQYACQRCTTLQDTNRIFTDAFDILAEHFEFCENKGRTVAFLRASSLIKSLPFPITAMKELEGLPWLGDQMKGIIEEILEEGKSYKVLEVMNEERYKSFKQFTSVFGVGLKTSDKWFRMGFRTLEEIKNEKELKLTKMQKCGLLYYEDITSYVSRAEAETTEQLIKSIVWKFVPDAIVTLTGGFRRGKKKGHDVDILITCARKGKEKNILHNTMSVLKNRGLLLFYNIIESTFDETKLPSRHVDALDHFQKCFTILKLPKRQMDIGNIIDPHECERKNWKAVRLDLVITPYEQYPYALLGWTGSRQFERDLRRYATHEKRMMLDNHGLYDKTKNNFLKANNEEDIFKQLGLDYLEPWERNA

SEQ ID NO: 30 - protein, 383 aa, synthetic construct
  REGION 1..383: note = B63 trunc wt (Notechis scutatus) tiger snake
SPSPVPGSQNVPAPSVDSISPYACQRRTTLKNYNQKFTDAFEILVENYEFNENKEFCLAFGRAASLLKCLPFTVVRVNDIEGLPWMGKQVREIIEDILEEGESSKVKAVLNDENYRSIKLFTSVFGVGLRTSEKWYRMGLRTLEEVKCNKNLTLTRMQKAGFFYYDDLISSVSKAEADAATQIVQDTVWKILPNAVVTLTGGFRRGKQTGHDVDFLITVPGSRQEEELLHPVIDIWKKQELLLYYDLIESTFENTKLPSRKVDALDHFQKCFAILKVHKERVNKGSAVQSNVFAEEGTKDWKAIRVDLVVTPFQHYAFALLGWTGSRQFERDLRRYATQEKKMMLDNHALYDKTKKIFLSAANEEEIFSHLGLDYLEPWERNA

SEQ ID NO: 31 - protein, 367 aa, synthetic construct
  REGION 1..367: note = F15 trunc wt (Salmo trutta) brown trout
TAAANVSQYACLRRTTTENHNKIFTDVLEELAENSEFNESKGPCLAFRRAASVLKSLPSAVHCLGAIQGLPCLGEHTKAVMEEILIFGRSFKVEEVQSDERYQALKLFTSVFGVGPKTAEKWYRRGLRSLKEILAEPNIQLNRMQRAGFLYYRDISKAVSKAEAKALSSIIEETAHWIAPDSILALTGGFRRGKEYGHDVDFLLTMPEMGKEEGLLLRVIDRLRDQGILLYCEHQDSTFDMSKLPSHRFEAMDHFEKCFLILRLEEGQVEGDGGLQKDPGESRGWRAVRVDLVAPPVDRYAFVLLGWTGSRQFERDLRRFASKERGMCLDNHALYDKTKKLFLPATSEEDIFAHLGLEYVEPWQRNA

SEQ ID NO: 32 - protein, 377 aa, synthetic construct
  REGION 1..377: note = F24 trunc wt (Electrophorus electricus) electric eel
SPSPVPGSQNVPAPSLPTVSQYACQRRTTLDNHNKVFTDALEVLIENYEFSDNKGACVGFRRAASVLKSLPKPLRCLKDMEGLPCLGDDTKAIIEEIYECGSSSRVENILSDEKYQTLKLFTSVFGVGPKTGEKWYRRGLRALEQVHSEPSIQLNKMQAAGFLYYEDISKPVSRAEAKAVGCIIEEVASCFSSSVTITLTGGFRRGKEFGHDVDFLLSIPEPGKEDGLLPAVIDRLRKQGILLYSDLQESTLQQWKRPSRCFDSMDHFQKCFLIVKLWTRLVEGHREDPSSQRDWKAVRVDLVVPPVDCYAFALLGWSGSTQFERDLRRFARLERRMLLDNHALYDKTTNTFLQAKTEEDIFAHLGLDYIEPWQRNA

SEQ ID NO: 33 - protein, 378 aa, synthetic construct
  REGION 1..378: note = F32 trunc wt (Anabas testudineus) walking fish
SPSPVPGSQNVPAPSVATVSQYACQRRTTTENNNKILTDAFEVLAESYELNQLEGPCLAFRRAASVLKSLPWAVQCLGATQGLPCLGEHTKALIEEILQYGHSFEVEKILSDERYQTLKLFTSVFGVGPKTAEKWYRRGLRSFSDILAEPSIQLNRMQQSGFLHYGDISRAVSKAEARALGNIIDEAVHAITPDGILALTGGFRRGKEFGHDVDFIVTTPEQGKEETLLPNIIDRLKEQGILLYSDYQTSTFDISKLPSHKFEAMDHFAKCFLILRLEGSLVDRGLNSTEGDSRGWRAVRVDLVSPPMERYAYALLGWTGSRQFERDLRRFARLEQHMLLDNHALYDKTKKEFLAATTERDIFAHLGLEYIEPWQRNA

SEQ ID NO: 34 - protein, 378 aa, synthetic construct
  REGION 1..378: note = F57 trunc wt (Poecilia reticulate) guppy
SPSPVPGSQNVPAPSVDKVSQYACQRRTTVENNNRIFTDAFEVLAENYEFNEIEGRCLAFRRAASVLKSLPWAVRSVGATLDLPCLGEHTTAVMKEILQYGRSFEVEKILSDERCQTLKLFTSVFGVGPKTAEKWYRRGLRSFSDVLAQPGIHLNRMQQSGFLHYGDISRAVSKAEARAVGNIIDEAVHVITPNAILALTGGFRRGKDFGHDVDFIVTTTELGKEKNLLISVIESLKKQGLLLFSDYQASTFDISKLPSHRFEAMDHFAKCFLILRLEGSRVEGGLQRAQADGRGWRAVRVDLVSPPADRFAFTMLGWTGSRMFERDLRRFARLERQMLLDNHALYDKTKKEFLTAATEKDIFDHLGLEYIEPWQRNA

SEQ ID NO: 35 - protein, 366 aa, synthetic construct
  REGION 1..366: note = N100 trunc wt (short Rattus norvegicus)
PLMQKISQYACQRRTTLNNHNQLFTDAFDILAENYEFRENEVSCLPFMRAASVLKSLSFPIVSMKDIEGIPCLGDKVKCVIEGIIEDGESSEVKAVLNDERYKSFKLFTSVFGVGLKTAEKWFRMGFRTLSKIKSDKSLRFTHMQKAGFLYYEDLVSCVNRAEAEAVSMLVKEAVVAFLPDALVTMTGGFRRGKMTGHDVDFLITSPEATEEEEQQLLHKVTNFWRQQGLLLYCDIIESTFEKFKLPSRKVDALDHFQKCFLILKLHRGLVRSEESGQQEGKDWKAIRVDLVMCPYERRAFALLGWTGSRQFERDLRRYATHERKMMLDNHALYDKTKRVFLEAESEEEIFAHLGLDYIEPWERNA

SEQ ID NO: 36 - protein, 379 aa, synthetic construct
  REGION 1..379: note = N100or trunk wt (long Rattus norvegicus)
SLSPVPGSQTVPPPLMQKISQYACQRRTTLNNHNQLFTDAFDILAENYEFRENEVSCLPFMRAASVLKSLSFPIVSMKDIEGIPCLGDKVKCVIEGIIEDGESSEVKAVLNDERYKSFKLFTSVFGVGLKTAEKWFRMGFRTLSKIKSDKSLRFTHMQKAGFLYYEDLVSCVNRAEAEAVSMLVKEAVVAFLPDALVTMTGGFRRGKMTGHDVDFLITSPEATEEEEQQLLHKVTNFWRQQGLLLYCDIIESTFEKFKLPSRKVDALDHFQKCFLILKLHRGLVRSEESGQQEGKDWKAIRVDLVMCPYERRAFALLGWTGSRQFERDLRRYATHERKMMLDNHALYDKTKRVFLEAESEEEIFAHLGLDYIEPWERNA

SEQ ID NO: 37 - protein, 379 aa, synthetic construct
  REGION 1..379: note = N14 trunc wt (Piliocolobus tephrosceles) monkey
SDSTNPGLPKTPPTAIQKISQYACQRRTTLNNCNQIFTDAFDILAENCEFRENEDSCVTFMRAASVLKSLPFTIISMKDTEGIPCLGSKVKCIIEEIIEDGESSEVKAVLNDERYQSFKLFTSVFGVGLKTSEKWFRMGFRTLSKVRSDESLKFTRMQRAGFLYYEDLVSCVTRAEAEAVSALVKEAVWAFLPDAFVTMTGGFRRGKKMGHDVDFLITSPGSTEDEEQQLLQKVMNLWEKKGLLLYYDLVESTFEKLRLPSRKVDALDHFQKCFLIFKLPLQRVDSDQSSWQGGKTWKAIRVDLVMCPYERRAFALLGWTGSRQFERDLRRYATHERKMILDNHALYDKTKRIFLKAESEEEIFAHLGLDYIEPWERNA

SEQ ID NO: 38 - protein, 379 aa, synthetic construct
  REGION 1..379: note = N27 trunc wt (Sus scrofa) pig
SASPSPGSQNTLPPAVKKISQYACQRRTTLNNCNHIFTDAFEVLAENYEFRENETFCLAFMRAASVLKSLPFTIISMKDTEGIPCLGDKVKCVIEEIIEDGESSEVKAVLNDERYQSFKLFTSVFGVGLKTSERWFRMGFRSLSKIRSDKTLKFTRMQKAGFLYYEDLVSCVTRAEAEAVGVLVKEAVQAFLPDAFVTMTGGFRRGKKMGHDVDFLITSPGSTDDEEQQLLPKVVNLWEREGLLLYCDLVESTLEKSKLPSRNVDALDHFQKCFLILKLHHQRVDSGMSSQQEGKTWKAIRVDLVMCPYELRAFALLGWTGSRQFERDLRRYATHERKMILDNHALYDKTKRIFLKAESEEEIFAHLGLDYLEPWERNA

SEQ ID NO: 39 - protein, 379 aa, synthetic construct
  REGION 1..379: note = N35 trunc wt (Panthera tigris altaica) Siberian tiger
YSASPNPELQKTPPLVKKIPLYACQRRTTLNNFNHVFTDAFEVLAENYEFKENEVSSATFMRAASVLKSLPFTIISMKDTEGIPCLGDKVKCVIEEIIEDGESSEVKAVLNDERYQSFKLFTSVFGVGLKTSEKWFRMGFRTLSKIKSDKTLKFTQMQKAGFLYYEDLVSCVTRAEAEAVGVLVKEAVWAFLPDAFVTMTGGFRRGKKIGHDVDFLITSPGSTDEEEEELLPKVINLWQRKELLLYYDLVESTFEKLKLPSRKVDALDHFQKCFLILKLHHQRVDSGKCSQQEGKTWKAIRVDLVMCPYERRAFALLGWTGSRQFERDLRRYATHERKMILDNHALYDKTKKIFLKAESEEEIFAHLGLDYIEPWERNA

SEQ ID NO: 40 - protein, 365 aa, synthetic construct
  REGION 1..365: note = N72 trunc wt (Bubalus bubalis) water buffalo
LAVKKISQYACQRKTTLNNYNHIFTDAFEILAENSEFKENEVSYVTFMRAASVLKSLPFTIISMKDTQGIPCLGDKVKCVIEEIIEDGESSEVKAVLNDERYQSFKLFTSVFGVGLKTSEKWFRMGFRSLSKITSDKTLKFTKMQKAGFLYYEDLVSCVTRAEAEAVGVLVKEAVWAFLPDAFITMTGGFRRGKKIGHDVDFLITSPGSAEDEEQLLPKVINLWEKKGLLLYYDLVESTFEKFKLPSRQVDTLDHFQKCFLILKLHHQRVDSGRSNQQEGKTWKAIRVDLVMCPYENRAFALLGWTGSRQFERDIRRYATHERKMMLDNHALYDKTKRVFLKAESEEEIFAHLGLDYIEPWERNA

SEQ ID NO: 41 - protein, 379 aa, synthetic construct
  REGION 1..379: note = N93or trunc wt (Marmota flaviventris) marmot
PDHSNSDPQRIPPPAVQTISQYACQRRTTLNNCNRVFTDAFDVLAENYEFRENESCSVVFMRAASVLKSLPFTIISMRDLEGIPCLEGKAKSIIEEIIEDGESSEVKAVLNDERYKSFKLFTSVFGVGLKTSEKWFRMGFRTLSKIRSDKSLKFTHMQKAGFLYYEDLVSCVTRAEAEAVSVLVKEAVWAFLPDAFITMTGGFRRGKNIGHDVDFLITSAEATEEEEQQLLHKVTNLWEKKGLLLYCDLVESTFEKLKTPSRKVDALDHFQKCFLILKLHHQRVDSDKASQQGGKNWKAIRVDLVMCPYERRAFALLGWTGSRQFERDLRRYATHERKMILDNHALYDKTKRIFLKAESEEEIFAHLGLDYIEPWERNA

SEQ ID NO: 42 - protein, 172 aa, synthetic construct
  REGION 1..172: note = N-terminal truncated WT mouse segment (B1)
NSSPSPVPGSQNVPAPAVKKISQYACQRRTTLNNYNQLFTDALDILAENDELRENEGSCLAFMRASSVLKSLPFPITSMKDTEGIPCLGDKVKSIIEGIIEDGESSEAKAVLNDERYKSFKLFTSVFGVGLKTAEKWFRMGFRTLSKIQSDKSLRFTQMQKAGFLYYEDLVS

SEQ ID NO: 43 - protein, 68 aa, synthetic construct
  REGION 1..68: note = C-terminal truncated WT mouse segment (B3)
RAFALLGWTGSRQFERDLRRYATHERKMMLDNHALYDRTKRVFLEAESEEEIFAHLGLDYIEPWERNA

SEQ ID NO: 44 - protein, 145 aa, synthetic construct
  REGION 1..145: note = B10 center segment wt (Serinus canaria)(canary)
CVSKAEADAVSLIVKNTVCTFLPDALVTITGGFRRGKNIGHDIDFLITNPGPREDDELLHKVIDLWKKQGLLLYCDIIESTFVKEQLPSRKIDAMDHFQKCFAILKLYQPRVDNSTCNTSKKLEMAEVKDWKAIRVDLVITPFEQ

SEQ ID NO: 45 - protein, 145 aa, synthetic construct
  REGION 1..145: note = B19center segment wt (Neopelma chrysocephalum)(saffron-crested neopelma)
CVSKAEADAVTLIVKNTVSTFLPDALVTITGGFRRGKKMGHDIDFLITNPGPREDDELLHKVVDLWKKQGLLLYCDIIESTFVEEQLPSRKVDAMDNFQKCFTILKLYQPGVDNSSYNMSKKSDMAEVKDWKAIRVDLVITPFEQ

SEQ ID NO: 46 - protein, 145 aa, synthetic construct
  REGION 1..145: note = B57 center segment wt (Alligator sinensis)
YVSKAEADAVSLLIKDTVCMFLPDALVTITGGFRRGKKTGHDVDFLITNPGPEEEKELLHKVVDLWEKQGLLLYYDVIESTFEKEKRPSRKVDALDHFQKCFAILKLHQQRRGNSNSNISKESDKAEVKDWKAIRVDLVISPFEQ

SEQ ID NO: 47 - protein, 145 aa, synthetic construct
  REGION 1..145: note = B63 center segment wt (Notechis scutatus) tiger snake
SVSKAEADAATQIVQDTVWKILPNAVVTLTGGFRRGKQTGHDVDFLITVPGSRQEEELLHPVIDIWKKQELLLYYDLIESTFENTKLPSRKVDALDHFQKCFAILKVHKERVNKGSAVQSNVFAEEGTKDWKAIRVDLVVTPFQH

SEQ ID NO: 48 - protein, 142 aa, synthetic construct
  REGION 1..142: note = F15 center segment wt (Salmo trutta) brown trout
AVSKAEAKALSSIIEETAHWIAPDSILALTGGFRRGKEYGHDVDFLLTMPEMGKEEGLLLRVIDRLRDQGILLYCEHQDSTFDMSKLPSHRFEAMDHFEKCFLILRLEEGQVEGDGGLQKDPGESRGWRAVRVDLVAPPVDR

SEQ ID NO: 49 - protein, 139 aa, synthetic construct
  REGION 1..139: note = F24center segment wt (Electrophorus electricus) electric eel
PVSRAEAKAVGCIIEEVASCFSSSVTITLTGGFRRGKEFGHDVDFLLSIPEPGKEDGLLPAVIDRLRKQGILLYSDLQESTLQQWKRPSRCFDSMDHFQKCFLIVKLWTRLVEGHREDPSSQRDWKAVRVDLVVPPVDC

SEQ ID NO: 50 - protein, 140 aa, synthetic construct
  REGION 1..140: note = F32 center segment wt (Anabas testudineus) walking fish
AVSKAEARALGNIIDEAVHAITPDGILALTGGFRRGKEFGHDVDFIVTTPEQGKEETLLPNIIDRLKEQGILLYSDYQTSTFDISKLPSHKFEAMDHFAKCFLILRLEGSLVDRGLNSTEGDSRGWRAVRVDLVSPPMER

SEQ ID NO: 51 - protein, 140 aa, synthetic construct
  REGION 1..140: note = F57 center segment wt (Poecilia reticulate) guppy
AVSKAEARAVGNIIDEAVHVITPNAILALTGGFRRGKDFGHDVDFIVTTTELGKEKNLLISVIESLKKQGLLLFSDYQASTFDISKLPSHRFEAMDHFAKCFLILRLEGSRVEGGLQRAQADGRGWRAVRVDLVSPPADR

SEQ ID NO: 52 - protein, 141 aa, synthetic construct
  REGION 1..141: note = N100 center segment wt (short Rattus norvegicus)
CVNRAEAEAVSMLVKEAVVAFLPDALVTMTGGFRRGKMTGHDVDFLITSPEATEEEEQQLLHKVTNFWRQQGLLLYCDIIESTFEKFKLPSRKVDALDHFQKCFLILKLHRGLVRSEESGQQEGKDWKAIRVDLVMCPYER

SEQ ID NO: 53 - protein, 141 aa, synthetic construct
  REGION 1..141: note = N14 center segment wt (Piliocolobus tephrosceles) monkey
CVTRAEAEAVSALVKEAVWAFLPDAFVTMTGGFRRGKKMGHDVDFLITSPGSTEDEEQQLLQKVMNLWEKKGLLLYYDLVESTFEKLRLPSRKVDALDHFQKCFLIFKLPLQRVDSDQSSWQGGKTWKAIRVDLVMCPYER

SEQ ID NO: 54 - protein, 141 aa, synthetic construct
  REGION 1..141: note = N27 center segment wt (Sus scrofa) pig
CVTRAEAEAVGVLVKEAVQAFLPDAFVTMTGGFRRGKKMGHDVDFLITSPGSTDDEEQQLLPKVVNLWEREGLLLYCDLVESTLEKSKLPSRNVDALDHFQKCFLILKLHHQRVDSGMSSQQEGKTWKAIRVDLVMCPYEL

SEQ ID NO: 55 - protein, 141 aa, synthetic construct
  REGION 1..141: note = N35 center segment wt (Panthera tigris altaica) Siberian tiger
CVTRAEAEAVGVLVKEAVWAFLPDAFVTMTGGFRRGKKIGHDVDFLITSPGSTDEEEEELLPKVINLWQRKELLLYYDLVESTFEKLKLPSRKVDALDHFQKCFLILKLHHQRVDSGKCSQQEGKTWKAIRVDLVMCPYER

SEQ ID NO: 56 - protein, 140 aa, synthetic construct
  REGION 1..140: note = N72 center segment wt (Bubalus bubalis) water buffalo
CVTRAEAEAVGVLVKEAVWAFLPDAFITMTGGFRRGKKIGHDVDFLITSPGSAEDEEQLLPKVINLWEKKGLLLYYDLVESTFEKFKLPSRQVDTLDHFQKCFLILKLHHQRVDSGRSNQQEGKTWKAIRVDLVMCPYEN

SEQ ID NO: 57 - protein, 141 aa, synthetic construct
  REGION 1..141: note = N93or center segment wt (Marmota flaviventris) marmot
CVTRAEAEAVSVLVKEAVWAFLPDAFITMTGGFRRGKNIGHDVDFLITSAEATEEEEQQLLHKVTNLWEKKGLLLYCDLVESTFEKLKTPSRKVDALDHFQKCFLILKLHHQRVDSDKASQQGGKNWKAIRVDLVMCPYER

SEQ ID NO: 58 - protein, 140 aa, synthetic construct
  REGION 1..140: note = Bovine center segment
CVTRAEAEAVGVLVKEAVWAFLPDAFVTMTGGFRRGKKIGHDVDFLITSPGSAEDEEQLLPKVINLWEKKGLLLYYDLVESTFEKFKLPSRQVDTLDHFQKCFLILKLHHQRVDSSKSNQQEGKTWKAIRVDLVMCPYEN

SEQ ID NO: 59 - protein, 140 aa, synthetic construct
  REGION 1..140: note = Human center segment
CVTRAEAEAVSVLVKEAVWAFLPDAFVTMTGGFRRGKKMGHDVDFLITSPGSTEDEEQLLQKVMNLWEKKGLLLYYDLVESTFEKLRLPSRKVDALDHFQKCFLIFKLPRQRVDSDQSSWQEGKTWKAIRVDLVLCPYER

SEQ ID NO: 60 - protein, 137 aa, synthetic construct
  REGION 1..137: note = Chicken center segment
CVSKAEADAVSSIVKNTVCTFLPDALVTITGGFRRGKKIGHDIDFLITSPGQREDDELLHKGLLLYCDIIESTFVKEQIPSRHVDAMDHFQKCFAILKLYQPRVDNSSYNMSKKCDMAEVKDWKAIRVDLVITPFEQ

SEQ ID NO: 61 - protein, 147 aa, synthetic construct
  REGION 1..147: note = Possum center segment
CVSKAEADAVSLLVQDAVWTFLPDALVTITGGFRRGKEFGHDVDFLITSPGAEKEQEDQLLQKVTNLWKKQGLLLYCDLIESTFEDLKLPSRKIDALDHFQKCFLILKLYHHKEDKRKWEMPTGSNESEAKSWKAIRVDLVVCPYDR

SEQ ID NO: 62 - protein, 141 aa, synthetic construct
  REGION 1..141: note = New center segment shrew
CVTRAEAEAVGVLVKEAVWAFLPDAIVTMTGGFRRGKKVGHDVDFLITSPEATEEQEQQLLHKVITFWEKEGLLLYCDLYESTFEKLKMPSRKVDALDHFQKCFLILKLHRECVDDGTSSQLQGKTWKAIRVDLVVCPYEC

SEQ ID NO: 63 - protein, 141 aa, synthetic construct
  REGION 1..141: note = center segment dog
CVTRAEAEAVGVLVKEAVGAFLPDAFVTMTGGFRRGKKMGHDVDFLITSPGSTDEDEEQLLPKVINLWERKGLLLYCDLVESTFEKLKLPSRKVDALDHFQKCFLILKLHHQRVDGGKCSQQEGKTWKAIRVDLVMCPYER

SEQ ID NO: 64 - protein, 141 aa, synthetic construct; identical to SEQ ID NO: 62
  REGION 1..141: note = center segment MOLE

SEQ ID NO: 65 - protein, 141 aa, synthetic construct
  REGION 1..141: note = Pika center segment
CVTRAEAEAVDVLVNEAVRAFLPDAFITMTGGFRRGKKIGHDVDFLITSPELTEEDEQQLLHKVMNLWEKKGLLLYHDLVESTFEKLKQPSRKVDALDHFQKCFLIFKLYHERVGGDRCRQPEGKDWKAIRVDLVMCPYEC

SEQ ID NO: 66 - protein, 144 aa, synthetic construct
  REGION 1..144: note = center segment HEDGEHOG
CVAKAEADAVSVLVQEAVWAFLPDAMVTMTGGFRRGKKLGHDVDFLITSPGATEEEEQQLLPKVINFWERKGLLLYHDLVESTFEKLKLPSRKVDALDHFQKCFLILKLHLQHVNGVGNSKTGQQEGKNWKAIRVDLVMCPYER

SEQ ID NO: 67 - protein, 141 aa, synthetic construct
  REGION 1..141: note = center segment tree shrew
CVTRAEAEAVGVLVKEAVGAFLPDALVTITGGFRRGKKTGHDVDFLITSPGSTEEKEEELLQKVLNLWEKKGLLLYYDLVESTFEKLKTPSRKVDALDHFPKCFLILKLHHQRVDGDKPSQQEGKSWKAIRVDLVMCPYER

SEQ ID NO: 68 - protein, 145 aa, synthetic construct
  REGION 1..145: note = center segment PLATYPUS
CVAKEEADAVYLIVKEAVRAFLPEALVTLTGGFRRGKKIGHDVDFLISDPESGQDEQLLPNIIKLWEKQELLLYYDLVESTFEKTKIPSRKVDAMDHFQKCFLILKLHHQKVDSGRYKPPPESKNHEAKNWKAIRVDLVMCPFEQ

SEQ ID NO: 69 - protein, 141 aa, synthetic construct
  REGION 1..141: note = center segment JERBOA
CVTRAEAEAVSVLVQQAVVAFLPDALVSMTGGFRRGKKIGHDVDFLITSPEATEEEEQQLLHKVTNFWEQKGLLLYCDHVESTFEKCKLPSRKVDALDHFQKCFLILKLYRERVDSVKSSQQEGKGWKAIRVDLVMCPYEC

SEQ ID NO: 70 - protein, 141 aa, synthetic construct
  REGION 1..141: note = center segment(Puma wildtype)
CVTRAEAEAVGVLVKEAVWAFLPDAFVTMTGGFRRGKKIGHDVDFLITIPGSTDEEEEQLLPKVINLWQRKELLLYYDLVESTFEKLKLPSRKVDALDHFQKCFLILKLHHQRVDSGKCSQQEGKTWKAIRVDLVMCPYER

SEQ ID NO: 71 - protein, 170 aa, synthetic construct
  REGION 1..170: note = N-terminal segment of M57 (N-terminus to VSC motif)
SPSPVPGSQNAPAPVVKKISQYACQRRTTLNNYNELFTRALDILAENDEFRENEESRDAFRRASSVLKSLPFPITSMKDTEGIPCLGDKVKRIIEEIIEDGESSEVKAVLNDERYKAFKLFTSVFGVGRKTAEKWFRMGFRTLEKIRSDKSLRFTQMQKAGFLYYEDLVS

SEQ ID NO: 72 - protein, 68 aa, synthetic construct
  REGION 1..68: note = C-terminal segment of M57
RAFALLGWTGSPQFNRDLRRYATHERKMMLDNHALYDKTKRVFLEAESEEEIFAHLGLDYIEPWERNA

SEQ ID NO: 73 - protein, 170 aa, synthetic construct
  REGION 1..170: note = N-terminal segment of M59
SPSPVPGSQNAPAPVVKKISQYACQRRTTLNNYNELFTRALDILAENDEFRENEESRDAFRRASSVLKSLPFPITSMKDTEGIPCLGDKVKRIIEEIIEDGESSEVKAVLNDERYKAFKLFTSVFGVGRKTAEKWFRMGFRTLEKIRSDKSLRFTQMQKAGFLYYEDLAE

SEQ ID NO: 74 - protein, 378 aa, synthetic construct
  REGION 1..378: note = mouse-bovine-pig chimera M57-N27-8-13C7 without His tag
SPSPVPGSQNAPAPVVKKISQYACQRRTTLNNYNELFTRALDILAENDEFRENEESRDAFRRASSVLKSLPFTITSMKDTEGIPCLGDKVKRIIEEIIEDGESSEVKAVLNDERYKAFKLFTSGFGVGRKTAEKWFRMGFRTLEKIRSDKTLKFTQMQKAGFLYYEDLASRVNRAEAEAIRVLVKEAVWAFLPDAFVTMTGGFRLGKKTGHDVDFLITSPGSTEDEEQLLHKVINLWEKKGLLLYYDLVESTFEKFKLPSRQVDTLDHFQKCFLILKLHHQRVDSSKSNQQEGKTWKAIRVDLVMCPYENRAFALLGWTGSPQFNRDLRRYATHERKQMLDNHALYDKTKRVFLEAESEEEIFRHLGLDYIEPWERNA

SEQ ID NO: 75 - protein, 364 aa, synthetic construct
  REGION 1..364: note = mouse-bovine chimera 46-557 without His tag
SEKKISEYACQRRTTLNNYNELFTRALDILAENDEFRENEESRDAFRRASSVLKSLPFPITSMKDTEGIPCLGDKVKRIIEEIIEDGESSEVKAVLNDERYKAFKLFTSVFGVGRKTAEKWFRMGFRTLEEIRSDKSLRFTQMQKAGFLYYEDLVSGVTRAEAEAVGVLVKEAVWAFLPDAFVTMTGGFRLGKKIGHDVDFLITSPGSAEDEEQLLPKVINLWEKKGLLLYYDLRESTFEKFKLPSRQVDTLDHFQKCFLILKLHHQRVDSSKSNQQEGKTWKAIRVDLVMCPYENRAFALLGWTGSPQFNRDLRRYATHERKMMLDNHALYDKTKRVFLEAESEEEIFAHLGLDYIEPWERNA

SEQ ID NO: 76 - protein, 364 aa, synthetic construct
  REGION 1..364: note = mouse-bovine chimera 46-342 without His tag
SEKKISEYACQRRTTLNNYNELFTRALDILAENDEFRENEESRDAFRRASSVLKSLPFPITSMKDTEGIPCLGDKVKRIIEEIIEDGESSEVKAVLNDERYKAFKLFTSVFGVGRKTAEKWFRMGFRTLEEIRSDKSLRFTQMQKAGFLYYEDLVSGVTRAEAEAVGVLVKEAVWAFLPDAFVTMTGGFRLGKKIGHDVDFLITSPGSAEDEEQLLPKVINLWEKKGLLLYYKLVESTFEKFKLPSRQVDTLDHFQKCFLILKLHHQRVDSSKSNQQEGKTWKAIRVDLVMCPYENRAFALLGWTGSPQFNRDLRRYATHERKMMLDNHALYDKTKRVFLEAESEEEIFAHLGLDYIEPWERNA

SEQ ID NO: 77 - protein, 364 aa, synthetic construct
  REGION 1..364: note = mouse-bovine chimera 46-571 without His tag
SEKKISEYACQRRTTLNNYNELFTRALDILAENDEFRENEESRDAFRRASSVLKSLPFPITSMKDTEGIPCLGDKVKRIIEEIIEDGESSEVKAVLNDERYKAFKLFTSVFGVGRKTAEKWFRMGFRTLEEIRSDKSLRFTQMQKAGFLYYEDLVSGVTRAEAEAVGVLVKEAVWAFLPDAFVTMTGGFRLGKKIGHDVDFLITSPGSAEDEEQLLPKVINLWEKKGLLLYYDLQESTFEKFKLPSRQVDTLDHFQKCFLILKLHHQRVDSSKSNQQEGKTWKAIRVDLVMCPYENRAFALLGWTGSPQFNRDLRRYATHERKMMLDNHALYDKTKRVFLEAESEEEIFAHLGLDYIEPWERNA

SEQ ID NO: 78 - protein, 390 aa, synthetic construct
  REGION 1..390: note = mouse-bovine chimera M92 without His tag
SENLYFQTGSSGSPSPVPGSQNVPAPVVKKISQYACQRRTTLNNYNQLFTDALDILAENDEFRENEDSRDAFRRASSVLKSLPFPITSMKDTEGIPCLGDKVKRIIEEIIEDGESSEVKAVLNDERYKAFKLFTSVFGVGRKTAEKWFRMGFRTLEKIRSDKSLRFTQMQKAGFLYYEDLAERVNRPEAEAIRMLVKEAVVTFLPDALVTMTGGFRLGKMTGHDVDFLITSPGSAEDEEQLLPKVINLWEKKGLLLYYDLVESTFEKFKLPSRQVDTLDHFQKCFLILKLHHQRVDSSKSNQQEGKTWKAIRVDLVMCPYENRAFALLGWTGSPQFNRDLRRYATHERKMMLDNHALYDKTKRVFLEAESEEEIFAHLGLDYIWPWERNA

SEQ ID NO: 79 - protein, 364 aa, synthetic construct
  REGION 1..364: note = mouse-bovine chimera M93 without His tag
SEKKISEYACQRRTTLNNYNEPFTRALDILAENDEFRENEESRDAFRRASSVLKSLPFPITSMKDTEGIPCLGDKVKRIIEEIIEDGESSEVKAVLNDERYKAFKLFTSVFGVGRKTAEKWFRMGFRTLEKIRSDKSLRFTQMQKAGFLYYEDLVSGVTRAEAEAVGVLVKEAVWAFLPDAFVTMTGGFRLGKKIGHDVDFLITSPGSAEDEEQLLPKVINLWEKKGLLLYYDLVESTFEKFKLPSRQVDTLDHFQKCFLILKLHHQRVDSSKSNQQEGKTWKAIRVDLVMCPYENRAFALLGWTGSPQFNRDLRRYATHERKMMLDNHALYDKTKRVFLEAESEEEIFAHLGLDYIEPWERNA

SEQ ID NO: 80 - protein, 364 aa, synthetic construct
  REGION 1..364: note = mouse-bovine chimera M94 without His tag
SEKKISEYACQRRTTLNNYNELFTRALDILAENDEFRENEESRDAFRRASSVLKSLPFPITSMKDTEGIPCLGDKVKRIIEEIIEDGESSEVKAVLNDERYKAFKLFTSVFGVGRKTAEKWFRMGFRTLEKIRSDKSLRFTQMQKAGFLYYEDLVSGVTRAEAEAVGVLVEEAVWAFLPDAFVTMTGGFRLGKKIGHDVDFLITSPGSAEDEEQLLPKVINLWEKKGLLLYYDLVESTFEKFKLPSRQVDTLDHFQKCFLILKLHHQRVDSSKSNQQEGKTWKAIRVDLVMCPYENRAFALLGWTGSPQFNRDLRRYATHERKMMLDNHALYDKTKRVFLEAESEEEIFAHLGLDYIEPWERNA

SEQ ID NO: 81 - protein, 364 aa, synthetic construct
  REGION 1..364: note = mouse-bovine chimera M88 without His tag
SEKKISEYACQRRTTLNNYNELFTRALDILAENDEFRENEESRDAFRRASSVLKSLPFPITSMKDTEGIPCLGDKVKRIIEEIIEDGESSEVKAVLNDERYKAFKLFTSVFGVGRKTAEKWFRMGFRTLEEIRSDKSLRFTQMQKAGFLYYEDLVSGVTRAEAEAVGVLVKEAVWAFLPDAFVTMTGGFRLGKKIGHDVDFLITSPGSAEDEEQLLPKVINLWEKKGLLLYYDLVESTLEKFKLPSRQVDRLDHFQKCFLILKLHRQRVDSSKSNQQEGKTWKAIRVDLVMCPYENRAFALLGWTGSPQFNRDLRRYATHERNMMLDNHALYDKTKRVFLEAESEEEIFAHLGLDYIWPWERNA

SEQ ID NO: 82 - protein, 154 aa, synthetic construct
  REGION 1..154: note = N-terminal segment of M77 to VSC motif
KKISEYACQRRTTLNNYNELFTRALDILAENDEFRENEESRDAFRRASSVLKSLPFPITSMKDTEGIPCLGDKVKRIIEEIIEDGESSEVKAVLNDERYKAFKLFTSVFGVGRKTAEKWFRMGFRTLEKIRSDKSLRFTQMQKAGFLYYEDLVS

SEQ ID NO: 83 - DNA, 12 bp, synthetic construct
  misc_feature 1..12: note = DNA INITIATOR
  misc_feature 11: note = "n" is deoxyinosine
  source 1..12: mol_type = other DNA
ttttttttttnt